European Patent Application EP 4 527 469 A2, published March 26, 2025. Title: BIOMIMETIC PEPTIDES DERIVED FROM BIOLOGICAL SOURCE AND THEIR USES IN RETARDING AGING AND IMPROVING SKIN. Applicant: TCI CO., LTD. Application EP. The sequence listing filed with the application follows.

SEQUENCE LISTING (15 sequences)

SEQ ID NO: 1 - skipped

SEQ ID NO: 2 - protein, 4 aa, synthetic construct
  REGION 1..4: note = Artificial peptide
RTCK

SEQ ID NO: 3 - protein, 4 aa, synthetic construct
  REGION 1..4: note = Artificial peptide
KSGR

SEQ ID NO: 4 - protein, 4 aa, synthetic construct
  REGION 1..4: note = Artificial peptide
KSGK

SEQ ID NO: 5 - protein, 4 aa, synthetic construct
  REGION 1..4: note = Artificial peptide
KYIK

SEQ ID NO: 6 - protein, 4 aa, synthetic construct
  REGION 1..4: note = Artificial peptide
KIFK

SEQ ID NO: 7 - protein, 4 aa, synthetic construct
  REGION 1..4: note = Artificial peptide
RPIK

SEQ ID NO: 8 - protein, 4 aa, synthetic construct
  REGION 1..4: note = Artificial peptide
KNAK

SEQ ID NO: 9 - protein, 5 aa, synthetic construct
  REGION 1..5: note = Artificial peptide
LKSGR

SEQ ID NO: 10 - protein, 5 aa, synthetic construct
  REGION 1..5: note = Artificial peptide
KIFKF

SEQ ID NO: 11 - protein, 5 aa, synthetic construct
  REGION 1..5: note = Artificial peptide
PRPIK

SEQ ID NO: 12 - protein, 6 aa, synthetic construct
  REGION 1..6: note = Artificial peptide
TKSGKF

SEQ ID NO: 13 - protein, 6 aa, synthetic construct
  REGION 1..6: note = Artificial peptide
VKNAKY

SEQ ID NO: 14 - protein, 7 aa, synthetic construct
  REGION 1..7: note = Artificial peptide
QKRRTCK

SEQ ID NO: 15 - protein, 8 aa, synthetic construct
  REGION 1..8: note = Artificial peptide
QRIKYIKP